European Patent Application EP 4 289 972 A1, published December 13, 2023. Title: METHOD FOR DETECTING METHICILLIN RESISTANT STAPHYLOCOCCUS AUREUS. Applicant: CONGEN Biotechnologie GmbH. Application EP. The sequence listing filed with the application follows.

SEQUENCE LISTING (52 sequences)

SEQ ID NO: 1 - DNA, 959 bp, synthetic construct
  source 1..959: mol_type = other DNA
ccgcttcataaagggattttgaatgtatcagaacatatgaggtttatgtgaattgctgttatgtttttaagaagcttatcataagtaatgaggttcatgatttttgacatagttagcctccgcagtctttcatttcaagtaaataatagcgaaatattctttatactgaatacttatagtgaagcaaagttctagctttgagaaaattctttctgcaactaaatatagtaaattacggtaaaatataaataagtacatattgaagaaaatgagacataatatattttataataggagggaatttcaaatgatagacaactttatgcaggtccttaaattaattaaagagaaacgtaccaataatgtagttaaaaaatctgattgggataaaggtgatctatataaaactttagtccatgataagttacccaagcagttaaaagtgcatataaaagaagataaatattcagttgtagggaaggttgctactgggaactatagtaaagttccttggatttcaatatatgatgagaatataacaaaagaaacaaaggatggatattatttggtatatctttttcatccggaaggagaaggcatatacttatctttgaatcaaggatggtcaaagataagtgatatgtttccgcgggataaaaatgctgcaaaacaaagagcattaactttatcttccgaactcaataaatatattacatcaaatgaatttaatactggaagattttattacgcagaaaataaagattcatcttatgatttaaaaaatgattatccatcaggatattctcatggatcaataagattcaaatattatgatttgaatgaaggattcacagaagaagatatgctagaggatttaaagaaatttttagaactatttaatgaattagcttcaaaagttacaaaaacatcctatgatagcttggtcaatagcatagacg

SEQ ID NO: 2 - DNA, 1246 bp, synthetic construct
  source 1..1246: mol_type = other DNA
tcatttcgccattttcctacattttataaccgccatttacatgaatcaaaggtaaaagaaaaagaaaaaagaaagcaacaaagagaagaagaaatagaaaaaaggagaatagcaaaagaagagcaagaaaagcgtgatgtttggattaaagagaatgtatttaaaattatagtaaatgaggaaggtaaacgaataattttttgtcctaaatgtggtagtgagaataatgtaactgctactacttggaacgtagatgaagctgaaaatagtgaggatattggaacatattttaagagaacttgtaatttatgcggacattctcaaaaatttaataaagataaccctaaaaaaatttatgaataggaataaagaattgatacattttctggataagtgaaaaagacaaattctattgaaataatatagaaattgtctttaatgttagaatttataaaacctcattatcaaccgatacgcagaagcatatcataaatgatgcggttttttcagccgcttcataaagggattttgaatgtatcagaacatatgaggtttatgtgaattgctgttatgtttttaagaagcttatcataagtaatgaggttcatgatttttgacatagttagcctccgcagtctttcatttcaagtaaataatagcgaaatattctttatactgaatacttatagtgaagcaaagttctagctttgagaaaattctttctgcaactaaatatagtaaattacggtaaaatataaataagtacatattgaagaaaatgagacataatatattttataataggagggaatttcaaatgatagacaactttatgcaggtccttaaattaattaaagagaaacgtaccaataatgtagttaaaaaatctgattgggataaaggtgatctatataaaactttagtccatgataagttacccaagcagttaaaagtgcatataaaagaagataaatattcagttgtagggaaggttgctactgggaactatagtaaagttccttggatttcaatatatgatgagaatataacaaaagaaacaaaggatggatattatttggtatatctttttcatccggaaggagaaggcatatacttatctttgaatcaaggatggtcaaagataagtgatatgtttccgcgggataaaaatgctgcaaaacaaagagcattaactttatcttccgaactcaataaatatattacatcaaatgaatttaatactgga

SEQ ID NO: 3 - DNA, 603 bp, synthetic construct
  source 1..603: mol_type = other DNA
gcaaaacctcgctttatagacgaattcgttctagagcaattgaacagtcatcttgataaattacccgaatatatagctacgatgactatgattgttcaagaatgtggaatgaggataagtgaattgtgcaccttgaaaaaaggctgtttattagaggacaaagatggagattactttttaaagtattatcaatggaaaatgaaaaaggagcatatagttccaatatctaaagaggtagttttacttattaaagttcgggaagataaagtttcagaggaatttccagatagtgaatacctctttccaagaaaagatggatcgccattaaaacaagaaacatttagaggcgaattaaataaattagcttatgagcaaagtatagtggataaattaggcgagatttatagattccatgcccatgcctttcgccattcagtaggaacaagaatgattaacaacggggtgccccagcatatcgtgcagaaatttttgggacatgaaagcccagaaatggcaagcagatacgctcatatctttgatcaaactctaaaaaatgaatttactaaatctgaagaaaaactggttaccaataatggagatgtg

SEQ ID NO: 4 - DNA, 1014 bp, synthetic construct
  source 1..1014: mol_type = other DNA
tctgtctttttcctttttgacgaaggcatgaaataagttcgaaattaatcatattagagttaatccatcgatagatggttttaaaacagatttggttttgtaatagacgacctacgatttgttcaggagaccagtggcattttaaataatatttaatgatattaccaagttctggagtaaatcgagtaggacgaccacaaagttttcttttggtttcataatttttttgagctgtttcagcttgatatgactgatttaaattattcctactaatttcacgtgagatagtagatacagatcgttttaatttacgtgcaatagatcttaaagaataattttcttgacgtaaaacctctatacgtgcgcgttcagttagtgtaagatggttatagctcatgttggcactccttgtatgtgtttttgtggttattaacatcttacaacaaagtgccaattatgggcattttttatgaatttttataggtgttgcacttaatattacaatccgtcgagtataaaaatgaaatagataaaattaaatctaaaattttaaatgaagaagacgagttagtaaaaaaatcattgatgttaacaatatttgtattatcggagagctatgttagttcattaattgtttctaatttacctgaaagagatgaaaatttaatagataaagcgtatgaaaaaattattcaacagtatataagtaaaaatatacgtacaagaaatggtagaaaagaactagtaaaaaatttttacaatacagatctaccagcaatacctcataccaaattgagagatgcccttgctcacgaaataaataaagttgatttaaaaaacaatcgttttaaatatgataatagtagaggtaatagaaatgaaaatattatagaagttagtattgacgaaataattaatgagttagaagaatggtttttaaatttagaatttccgtaaaaacctcatcatcaaccgataagcagaagcgtatcataaatgatgcggttttttcag

SEQ ID NO: 5 - DNA, 754 bp, synthetic construct
  source 1..754: mol_type = other DNA
tggtcatgcgaaaaaccaaacttgttaaacgttgcagtgacaagagctaagaaagagttttatgtaattggcgacatgcaaagaatacagatgaaaccattttatgagacgatttttaaagaaagaaatgtaaaatgaaattgaaataacagtattacttgatacttaattatcgagcaatttatacattttaaaaggagcaaaattgaataatgaagaaatttaacaactggatattaaatgcaataagtggatctcaaacagacaagaatgaaacaactgaagaattaaaaggggcaaaatttatcattttatatgcatattcaatgctcgttttgcttgcgttagtaatttctaacatattcattcacattttggagcctaaactatcaattaccactcaaatcatcatcgttttgattttaattgaaacactaattggactgcgtttcttgaaagcgtacgatgttaagcgtggcaaagataaagaaaataagaaaaatagtaaggatttcgttaaactaaaatcaattttagtagcaattttatttacatcattggcgctgacagcaggcactgtagctgatatatacggtttcactgacttaggaaatactagaagtgatttaatcgtttggagcataggtggtattatatttggcctcgtatgttacacaatggaagataaaaaataacgataaggagctggcgattataaagctagctccttttttaacttatgtaaatggcggtt

SEQ ID NO: 6 - DNA, 477 bp, synthetic construct
  source 1..477: mol_type = other DNA
aaaagacctgatattgtgttattcataaatggattaccagtagtggtaattgaactgaaaaattctacaaatgaatctgttggtattgaagacgggtatcatcagatagaaacttataaaatgagaactccacaattatttaatcataatgcagtattagttacgagtgatggtataaatacaaaagctggttctttaactgctgagtatgatcgttttatgacttggcgtactaaagatggaaaaactgaagattcatcaacatttcgtagtttagatatattgattcacggtatgttaaataaagaggtactattagatttaattcgtcattttgttttgttccaagatgatggtaaaggaaatatagttaaaatattagctgcatatcatcaatattatgcggttaataaagctgttgatcgtgctatggaagcaacatctgaacatggtgatggtaagggcggcgttatttgg

SEQ ID NO: 7 - DNA, 22 bp, synthetic construct
  source 1..22: mol_type = other DNA
ttccgtaaaaacctcatcatca

SEQ ID NO: 8 - DNA, 25 bp, synthetic construct
  source 1..25: mol_type = other DNA
cctacattttataaccgccatttac

SEQ ID NO: 9 - DNA, 23 bp, synthetic construct
  source 1..23: mol_type = other DNA
ctatggaagcaacatctgaacat

SEQ ID NO: 10 - DNA, 27 bp, synthetic construct
  source 1..27: mol_type = other DNA
aaacctcatatgttctgatacattcaa

SEQ ID NO: 11 - DNA, 25 bp, synthetic construct
  source 1..25: mol_type = other DNA
acattctctttaatccaaacatcac

SEQ ID NO: 12 - DNA, 23 bp, synthetic construct
  source 1..23: mol_type = other DNA
cattccacattcttgaacaatca

SEQ ID NO: 13 - DNA, 26 bp, synthetic construct
  source 1..26: mol_type = other DNA
accgataagcagaagcgtatcataaa

SEQ ID NO: 14 - DNA, 26 bp, synthetic construct
  source 1..26: mol_type = other DNA
aagaaaaagaaaaaagaaagcaacaa

SEQ ID NO: 15 - DNA, 19 bp, synthetic construct
  source 1..19: mol_type = other DNA
acgccgcccttaccatcac

SEQ ID NO: 16 - DNA, 110 bp, synthetic construct
  source 1..110: mol_type = other DNA
ttccgtaaaaacctcatcatcaaccgataagcagaagcgtatcataaatgatgcggttttttcagccgcttcataaagggattttgaatgtatcagaacatatgaggttt

SEQ ID NO: 17 - DNA, 143 bp, synthetic construct
  source 1..143: mol_type = other DNA
cctacattttataaccgccatttacatgaatcaaaggtaaaagaaaaagaaaaaagaaagcaacaaagagaagaagaaatagaaaaaaggagaatagcaaaagaagagcaagaaaagcgtgatgtttggattaaagagaatgt

SEQ ID NO: 18 - DNA, 161 bp, synthetic construct
  source 1..161: mol_type = other DNA
ctatggaagcaacatctgaacatggtgatggtaagggcggcgttatttgggcaaaacctcgctttatagacgaattcgttctagagcaattgaacagtcatcttgataaattacccgaatatatagctacgatgactatgattgttcaagaatgtggaatg

SEQ ID NO: 19 - DNA, 25 bp, synthetic construct
  source 1..25: mol_type = other DNA
agtactagccatattaatgcctcac

SEQ ID NO: 20 - DNA, 26 bp, synthetic construct
  source 1..26: mol_type = other DNA
cgtatctataataatgaatcgcctac

SEQ ID NO: 21 - DNA, 33 bp, synthetic construct
  source 1..33: mol_type = other DNA
  modified_base 19: mod_base = i
cttaatcaatttcaaaatnagttatatacaact

SEQ ID NO: 22 - DNA, 21 bp, synthetic construct
  source 1..21: mol_type = other DNA
gcggctgaaaaaaccgcatca

SEQ ID NO: 23 - DNA, 34 bp, synthetic construct
  source 1..34: mol_type = other DNA
caatcctttttatatttaaaataaattatacaca

SEQ ID NO: 24 - DNA, 32 bp, synthetic construct
  source 1..32: mol_type = other DNA
cttaatctttacttgtacctaaattatcaaac

SEQ ID NO: 25 - DNA, 29 bp, synthetic construct
  source 1..29: mol_type = other DNA
attattaattaatctgattttcactcttc

SEQ ID NO: 26 - DNA, 29 bp, synthetic construct
  source 1..29: mol_type = other DNA
catctcattaaatttttaaattatacaca

SEQ ID NO: 27 - DNA, 35 bp, synthetic construct
  source 1..35: mol_type = other DNA
ctttatgataatagactttataatataaatacaca

SEQ ID NO: 28 - DNA, 22 bp, synthetic construct
  source 1..22: mol_type = other DNA
caggtagttttaccttcccacc

SEQ ID NO: 29 - DNA, 29 bp, synthetic construct
  source 1..29: mol_type = other DNA
  modified_base 24: mod_base = i
taaatcccttccttttatattatncacaa

SEQ ID NO: 30 - DNA, 29 bp, synthetic construct
  source 1..29: mol_type = other DNA
gagtcacctcatattatattttttacaac

SEQ ID NO: 31 - DNA, 26 bp, synthetic construct
  source 1..26: mol_type = other DNA
ctcgtaatttaccttgttcattaaac

SEQ ID NO: 32 - DNA, 30 bp, synthetic construct
  source 1..30: mol_type = other DNA
taagtattcagtataaagaatatttcgcta

SEQ ID NO: 33 - DNA, 21 bp, synthetic construct
  source 1..21: mol_type = other DNA
tccccataaaaaaaccttcct

SEQ ID NO: 34 - DNA, 37 bp, synthetic construct
  source 1..37: mol_type = other DNA
aatatatcaaaatttagtaataattaatattgcatac

SEQ ID NO: 35 - DNA, 19 bp, synthetic construct
  source 1..19: mol_type = other DNA
gatcaaacggcctgctcaa

SEQ ID NO: 36 - DNA, 19 bp, synthetic construct
  source 1..19: mol_type = other DNA
gatcaaatggcctgctcaa

SEQ ID NO: 37 - DNA, 22 bp, synthetic construct
  source 1..22: mol_type = other DNA
tcaattaacacaacccgcatca

SEQ ID NO: 38 - DNA, 23 bp, synthetic construct
  source 1..23: mol_type = other DNA
cagcaaaatgacattcccacatc

SEQ ID NO: 39 - DNA, 82 bp, synthetic construct
  source 1..82: mol_type = other DNA
tcattcagcaaaatgacattcccacatcaaatgatgcgggttgtgttaattgcacaagtgtacagagcatttaagattatgc

SEQ ID NO: 40 - DNA, 132 bp, synthetic construct
  source 1..132: mol_type = other DNA
gatcaaacggcctgcacaaggacgtcttacaacgtagtaactacgcactatcattcagcaaaatgacattcccacatcaaatgatgcgggttgtgttaattgagcaagtgtatagagcatttaagattatgc

SEQ ID NO: 41 - DNA, 132 bp, synthetic construct
  source 1..132: mol_type = other DNA
gatcaaacggcctgcacaaggacgtcttacaacgcagtaactacgcactatcattcagcaaaatgacattcccacatcaaatgatgcgggttgtattaattgagcaagtgtacagagcatttaagattatgc

SEQ ID NO: 42 - DNA, 500 bp, synthetic construct
  source 1..500: mol_type = other DNA
gtggagaggcgtatcacaaataaaactaaaaatggagtaactattaatatagtataaattcaatatggtgataaaaacagcaaaaaaataaaatataacatcataaaggtgatgtgaatatattatacaaaaggggaatataatgttggaattaattactgatttttcaaaaaagtcttttaaaaattacagtatgaaggaagaattaaaattcaatgctataaatataatatacggagttaatgggaggggaaaaacttcattagctagaggtattaaagaaataatagaagaaaataatccagatagcttgaggtatttttacactgattatattcatgaacttcttttactagaagattccaataaatttaaaggggtaaaagcgacatttggtacaaaaaatgtagaaattgaaaataaaataatcaagctgaaaaatgaagttgttgatatgacggatactaaaaagttactagttgagaagagaaggaagttaa

SEQ ID NO: 43 - DNA, 500 bp, synthetic construct
  source 1..500: mol_type = other DNA
gtggagaggcgtatcataagtaggggtagtattagccaatttaataaataaagaggtgacagaatggacaatcacataagaatttttgataatttatttcaaagtaatatttcaaaattccaaaaccttactagtaaatcatacattataagaaatgataatgaaaagaatagttatcttcctatggttcaagagataagagagttgtttggaaaagagggagaaattttttctaaaagtataggaacacatcctgacttttttggaatagaaaatactaatgaataccagtacatttgttccctgtttgtagatatatctgggtctacaaagctagctttgaaatatagtttggataaagttaaactttataaaaatgcgataatttctagtgctatagaaatatttcgtgcatttgacggtcatattcatagaatacaaggagatgcggtgcttgtttattttggacataaagaactggaaaaaagtgatgcaataat

SEQ ID NO: 44 - DNA, 500 bp, synthetic construct
  source 1..500: mol_type = other DNA
gaggagaggcgtatcataagtagaagggggattagccaatttaataaataaaggggtgacagaatggacaatcacataaaaattttgacaatttatttcaaagtaatatttcaaaattccaaaatctttctagtaaatcatacattattagaaatgatactgaaaagaatagttatcttcctatggttcaagagataagagagttgtttggaaaagaaggagaaattttttctaaaagtataggaacacatcctgacttttttgaaatagaaaacactaatgaataccagtacatttgttccctttttgtagatatatctgggtctacaaaactagctttgaaatatagtttggataaagttaaactttataaaaatgcgataatttctagtgctatagaaatatttcgtgcatttgacggtcatattcatagaatacaaggagatgcggtgcttgtttattttggacataaagaactggaaaaaagtgatgcaataatt

SEQ ID NO: 45 - DNA, 29 bp, synthetic construct
  source 1..29: mol_type = other DNA
cgattataaagctagctccttttttaact

SEQ ID NO: 46 - DNA, 1973 bp, synthetic construct
  source 1..1973: mol_type = other DNA
tctgtctttttcctttttgacgaaggcatgaaataagttcgaaattaatcatattagagttaatccatcgatagatggttttaaaacagatttggttttgtaatagacgacctacgatttgttcaggagaccagtggcattttaaataatatttaatgatattaccaagttctggagtaaatcgagtaggacgaccacaaagttttcttttggtttcataatttttttgagctgtttcagcttgatatgactgatttaaattattcctactaatttcacgtgagatagtagatacagatcgttttaatttacgtgcaatagatcttaaagaataattttcttgacgtaaaacctctatacgtgcgcgttcagttagtgtaagatggttatagctcatgttggcactccttgtatgtgtttttgtggttattaacatcttacaacaaagtgccaattatgggcattttttatgaatttttataggtgttgcacttaatattacaatccgtcgagtataaaaatgaaatagataaaattaaatctaaaattttaaatgaagaagacgagttagtaaaaaaatcattgatgttaacaatatttgtattatcggagagctatgttagttcattaattgtttctaatttacctgaaagagatgaaaatttaatagataaagcgtatgaaaaaattattcaacagtatataagtaaaaatatacgtacaagaaatggtagaaaagaactagtaaaaaatttttacaatacagatctaccagcaatacctcataccaaattgagagatgcccttgctcacgaaataaataaagttgatttaaaaaacaatcgttttaaatatgataatagtagaggtaatagaaatgaaaatattatagaagttagtattgacgaaataattaatgagttagaagaatggtttttaaatttagaatttccgtaaaaacctcatcatcaaccgataagcagaagcgtatcataaatgatgcggttttttcagccgcttcataaagggattttgaatgtatcagaacatatgaggtttatgtgaattgctgttatgtttttaagaagcttatcataagtaatgaggttcatgatttttgacatagttagcctccgcagtctttcatttcaagtaaataatagcgaaatattctttatactgaatacttatagtgaagcaaagttctagctttgagaaaattctttctgcaactaaatatagtaaattacggtaaaatataaataagtacatattgaagaaaatgagacataatatattttataataggagggaatttcaaatgatagacaactttatgcaggtccttaaattaattaaagagaaacgtaccaataatgtagttaaaaaatctgattgggataaaggtgatctatataaaactttagtccatgataagttacccaagcagttaaaagtgcatataaaagaagataaatattcagttgtagggaaggttgctactgggaactatagtaaagttccttggatttcaatatatgatgagaatataacaaaagaaacaaaggatggatattatttggtatatctttttcatccggaaggagaaggcatatacttatctttgaatcaaggatggtcaaagataagtgatatgtttccgcgggataaaaatgctgcaaaacaaagagcattaactttatcttccgaactcaataaatatattacatcaaatgaatttaatactggaagattttattacgcagaaaataaagattcatcttatgatttaaaaaatgattatccatcaggatattctcatggatcaataagattcaaatattatgatttgaatgaaggattcacagaagaagatatgctagaggatttaaagaaatttttagaactatttaatgaattagcttcaaaagttacaaaaacatcctatgatagcttggtcaatagcatagacg

SEQ ID NO: 47 - DNA, 582 bp, synthetic construct
  source 1..582: mol_type = other DNA
tcattcagcaaaatgacattcccacatcaaatgatgcgggttgtgttaattgcacaagtgtacagagcatttaagattatgcgtggagaggcgtatcacaaataaaactaaaaatggagtaactattaatatagtataaattcaatatggtgataaaaacagcaaaaaaataaaatataacatcataaaggtgatgtgaatatattatacaaaaggggaatataatgttggaattaattactgatttttcaaaaaagtcttttaaaaattacagtatgaaggaagaattaaaattcaatgctataaatataatatacggagttaatgggaggggaaaaacttcattagctagaggtattaaagaaataatagaagaaaataatccagatagcttgaggtatttttacactgattatattcatgaacttcttttactagaagattccaataaatttaaaggggtaaaagcgacatttggtacaaaaaatgtagaaattgaaaataaaataatcaagctgaaaaatgaagttgttgatatgacggatactaaaaagttactagttgagaagagaaggaagttaa

SEQ ID NO: 48 - DNA, 2000 bp, synthetic construct
  source 1..2000: mol_type = other DNA
tggtcatgcgaaaaaccaaacttgttaaacgttgcagtgacaagagctaagaaagagttttatgtaattggcgacatgcaaagaatacagatgaaaccattttatgagacgatttttaaagaaagaaatgtaaaatgaaattgaaataacagtattacttgatacttaattatcgagcaatttatacattttaaaaggagcaaaattgaataatgaagaaatttaacaactggatattaaatgcaataagtggatctcaaacagacaagaatgaaacaactgaagaattaaaaggggcaaaatttatcattttatatgcatattcaatgctcgttttgcttgcgttagtaatttctaacatattcattcacattttggagcctaaactatcaattaccactcaaatcatcatcgttttgattttaattgaaacactaattggactgcgtttcttgaaagcgtacgatgttaagcgtggcaaagataaagaaaataagaaaaatagtaaggatttcgttaaactaaaatcaattttagtagcaattttatttacatcattggcgctgacagcaggcactgtagctgatatatacggtttcactgacttaggaaatactagaagtgatttaatcgtttggagcataggtggtattatatttggcctcgtatgttacacaatggaagataaaaaataacgataaggagctggcgattataaagctagctccttttttaacttatgtaaatggcggtttcatttcgccattttcctacattttataaccgccatttacatgaatcaaaggtaaaagaaaaagaaaaaagaaagcaacaaagagaagaagaaatagaaaaaaggagaatagcaaaagaagagcaagaaaagcgtgatgtttggattaaagagaatgtatttaaaattatagtaaatgaggaaggtaaacgaataattttttgtcctaaatgtggtagtgagaataatgtaactgctactacttggaacgtagatgaagctgaaaatagtgaggatattggaacatattttaagagaacttgtaatttatgcggacattctcaaaaatttaataaagataaccctaaaaaaatttatgaataggaataaagaattgatacattttctggataagtgaaaaagacaaattctattgaaataatatagaaattgtctttaatgttagaatttataaaacctcattatcaaccgatacgcagaagcatatcataaatgatgcggttttttcagccgcttcataaagggattttgaatgtatcagaacatatgaggtttatgtgaattgctgttatgtttttaagaagcttatcataagtaatgaggttcatgatttttgacatagttagcctccgcagtctttcatttcaagtaaataatagcgaaatattctttatactgaatacttatagtgaagcaaagttctagctttgagaaaattctttctgcaactaaatatagtaaattacggtaaaatataaataagtacatattgaagaaaatgagacataatatattttataataggagggaatttcaaatgatagacaactttatgcaggtccttaaattaattaaagagaaacgtaccaataatgtagttaaaaaatctgattgggataaaggtgatctatataaaactttagtccatgataagttacccaagcagttaaaagtgcatataaaagaagataaatattcagttgtagggaaggttgctactgggaactatagtaaagttccttggatttcaatatatgatgagaatataacaaaagaaacaaaggatggatattatttggtatatctttttcatccggaaggagaaggcatatacttatctttgaatcaaggatggtcaaagataagtgatatgtttccgcgggataaaaatgctgcaaaacaaagagcattaactttatcttccgaactcaataaatatattacatcaaatgaatttaatactgga

SEQ ID NO: 49 - DNA, 632 bp, synthetic construct
  source 1..632: mol_type = other DNA
gatcaaacggcctgcacaaggacgtcttacaacgtagtaactacgcactatcattcagcaaaatgacattcccacatcaaatgatgcgggttgtgttaattgagcaagtgtatagagcatttaagattatgcgtggagaggcgtatcataagtaggggtagtattagccaatttaataaataaagaggtgacagaatggacaatcacataagaatttttgataatttatttcaaagtaatatttcaaaattccaaaaccttactagtaaatcatacattataagaaatgataatgaaaagaatagttatcttcctatggttcaagagataagagagttgtttggaaaagagggagaaattttttctaaaagtataggaacacatcctgacttttttggaatagaaaatactaatgaataccagtacatttgttccctgtttgtagatatatctgggtctacaaagctagctttgaaatatagtttggataaagttaaactttataaaaatgcgataatttctagtgctatagaaatatttcgtgcatttgacggtcatattcatagaatacaaggagatgcggtgcttgtttattttggacataaagaactggaaaaaagtgatgcaataat

SEQ ID NO: 50 - DNA, 1080 bp, synthetic construct
  source 1..1080: mol_type = other DNA
aaaagacctgatattgtgttattcataaatggattaccagtagtggtaattgaactgaaaaattctacaaatgaatctgttggtattgaagacgggtatcatcagatagaaacttataaaatgagaactccacaattatttaatcataatgcagtattagttacgagtgatggtataaatacaaaagctggttctttaactgctgagtatgatcgttttatgacttggcgtactaaagatggaaaaactgaagattcatcaacatttcgtagtttagatatattgattcacggtatgttaaataaagaggtactattagatttaattcgtcattttgttttgttccaagatgatggtaaaggaaatatagttaaaatattagctgcatatcatcaatattatgcggttaataaagctgttgatcgtgctatggaagcaacatctgaacatggtgatggtaagggcggcgttatttgggcaaaacctcgctttatagacgaattcgttctagagcaattgaacagtcatcttgataaattacccgaatatatagctacgatgactatgattgttcaagaatgtggaatgaggataagtgaattgtgcaccttgaaaaaaggctgtttattagaggacaaagatggagattactttttaaagtattatcaatggaaaatgaaaaaggagcatatagttccaatatctaaagaggtagttttacttattaaagttcgggaagataaagtttcagaggaatttccagatagtgaatacctctttccaagaaaagatggatcgccattaaaacaagaaacatttagaggcgaattaaataaattagcttatgagcaaagtatagtggataaattaggcgagatttatagattccatgcccatgcctttcgccattcagtaggaacaagaatgattaacaacggggtgccccagcatatcgtgcagaaatttttgggacatgaaagcccagaaatggcaagcagatacgctcatatctttgatcaaactctaaaaaatgaatttactaaatctgaagaaaaactggttaccaataatggagatgtg

SEQ ID NO: 51 - DNA, 632 bp, synthetic construct
  source 1..632: mol_type = other DNA
gatcaaacggcctgcacaaggacgtcttacaacgcagtaactacgcactatcattcagcaaaatgacattcccacatcaaatgatgcgggttgtattaattgagcaagtgtacagagcatttaagattatgcgaggagaggcgtatcataagtagaagggggattagccaatttaataaataaaggggtgacagaatggacaatcacataaaaattttgacaatttatttcaaagtaatatttcaaaattccaaaatctttctagtaaatcatacattattagaaatgatactgaaaagaatagttatcttcctatggttcaagagataagagagttgtttggaaaagaaggagaaattttttctaaaagtataggaacacatcctgacttttttgaaatagaaaacactaatgaataccagtacatttgttccctttttgtagatatatctgggtctacaaaactagctttgaaatatagtttggataaagttaaactttataaaaatgcgataatttctagtgctatagaaatatttcgtgcatttgacggtcatattcatagaatacaaggagatgcggtgcttgtttattttggacataaagaactggaaaaaagtgatgcaataatt

SEQ ID NO: 52 - DNA, 20 bp, synthetic construct
  source 1..20: mol_type = other DNA
taatacgactcactataggg